European Patent Specification EP 4 440 621 B1, published February 4, 2026. Title: Peptide-drug conjugates for treatment of neurodegenerative diseases. Applicant: University of Copenhagen. The sequence listing filed with the application follows.

SEQUENCE LISTING (9 sequences)

SEQ ID NO: 1 - protein, 40 aa, Homo sapiens
  VARIANT 2: note = D-alanine, D-serine, alpha-aminoisobutyric acid, N-methyl-serine, glycine, or valine
  VARIANT 40: note = L-penicillamine or L-homocysteine
HAEGTFTSDVSSYLEEQAAKEFIAWLVKGGPSSGAPPPSC

SEQ ID NO: 2 - protein, 31 aa, Homo sapiens
HAEGTFTSDVSSYLEGQAAKEFIAWLVKGRG

SEQ ID NO: 3 - protein, 39 aa, Homo sapiens
HGEGTFTSDLSKQMEEEAVRLFIEWLKNGGPSSGAPPPS

SEQ ID NO: 4 - protein, 42 aa, Homo sapiens
YAEGTFISDYSIAMDKIHQQDFVNWLLAQKGKKNDWKHNITQ

SEQ ID NO: 5 - protein, 40 aa, Homo sapiens
  VARIANT 2: note = alpha-aminoisobutyric acid
  VARIANT 20: note = alpha-aminoisobutyric acid
  VARIANT 40: note = L-Penicillamine
YGEGTFTSDYSIYLDKQAAKEFVNWLLAGGPSSGAPPPSC

SEQ ID NO: 6 - protein, 39 aa, Homo sapiens
  VARIANT 2: note = D-alanine, D-serine, alpha-aminoisobutyric acid, N-methyl-serine, glycine, or valine
  VARIANT 13: note = D-alanine, D-serine, alpha-aminoisobutyric acid, N-methyl-serine, glycine, or valine
YAEGTFTSDYSIALDKIAQKAFVQWLIAGGPSSGAPPPS

SEQ ID NO: 7 - protein, 39 aa, Homo sapiens
  VARIANT 2: note = D-alanine, D-serine, alpha-aminoisobutyric acid, N-methyl-serine, glycine, or valine
HAQGTFTSDKSKYLDERAAQDFVQWLLDGGPSSGAPPPS

SEQ ID NO: 8 - protein, 40 aa, Homo sapiens
  VARIANT 2: note = D-alanine, D-serine, alpha-aminoisobutyric acid, N-methyl-serine, glycine, or valine
  VARIANT 1: note = X is any natural or synthetic amino acid
  VARIANT 10: note = X is any natural or synthetic amino acid
  VARIANT 12: note = X is any natural or synthetic amino acid
  VARIANT 15: note = X is any natural or synthetic amino acid
  VARIANT 16: note = X is any natural or synthetic amino acid
  VARIANT 23: note = X is any natural or synthetic amino acid
  VARIANT 24: note = X is any natural or synthetic amino acid
  VARIANT 27: note = X is any natural or synthetic amino acid
  VARIANT 28: note = X is any natural or synthetic amino acid
  VARIANT 40: note = L-penicillamine or L-homocysteine
XAEGTFTSDXSXYLXXQAAKEFXXWLXXGGPSSGAPPPSC

SEQ ID NO: 9 - protein, 10 aa, Homo sapiens
GPSSGAPPPS